European Patent Application EP 4 299 182 A1, published January 3, 2024. Title: Method for pulverization, Method for producing polymer block and apparatus for pulverization. Applicant: FUJIFILM CORPORATION. The sequence listing filed with the application follows.

SEQUENCE LISTING (1 sequence)

SEQ ID NO: 1 - protein, 571 aa, Artificial
  CBE3
GAPGAPGLQGAPGLQGMPGERGAAGLPGPKGERGDAGPKGADGAPGAPGLQGMPGERGAAGLPGPKGERGDAGPKGADGAPGKDGVRGLAGPIGPPGERGAAGLPGPKGERGDAGPKGADGAPGKDGVRGLAGPIGPPGPAGAPGAPGLQGMPGERGAAGLPGPKGERGDAGPKGADGAPGKDGVRGLAGPPGAPGLQGAPGLQGMPGERGAAGLPGPKGERGDAGPKGADGAPGAPGLQGMPGERGAAGLPGPKGERGDAGPKGADGAPGKDGVRGLAGPIGPPGERGAAGLPGPKGERGDAGPKGADGAPGKDGVRGLAGPIGPPGPAGAPGAPGLQGMPGERGAAGLPGPKGERGDAGPKGADGAPGKDGVRGLAGPPGAPGLQGAPGLQGMPGERGAAGLPGPKGERGDAGPKGADGAPGAPGLQGMPGERGAAGLPGPKGERGDAGPKGADGAPGKDGVRGLAGPIGPPGERGAAGLPGPKGERGDAGPKGADGAPGKDGVRGLAGPIGPPGPAGAPGAPGLQGMPGERGAAGLPGPKGERGDAGPKGADGAPGKDGVRGLAGPPG